European Patent Specification EP 3 532 092 B1, published April 29, 2026. Title: Immunoglobulins and Uses Thereof. Applicant: Janssen Pharmaceutica NV. The sequence listing filed with the application follows.

SEQUENCE LISTING (27 sequences)

SEQ ID NO: 1 - protein, 34 aa, Homo sapiens
IKPEAPGEDASPEELNRYYASLRHYLNLVTRQRY

SEQ ID NO: 2 - protein, 35 aa, Artificial Sequence
  Compound 1
  Ala (1)..(1): Ala with chemical modification as described in the specification
  Lys (10)..(10): Lys with chemical modification as described in the specification
  Cys (30)..(30): Cys, wherein cys is homocysteine with chemical modification as described in the specification
  Arg (34)..(34): Arg with chemical modification as described in the specification
AIKPEAPGEKASPEELNRYYASLRHYLNLCTRQRY

SEQ ID NO: 3 - protein, 107 aa, Homo sapiens
EIVLTQSPATLSLSPGERATLSCRASQSVSSYLAWYQQKPGQAPRLLIYDASNRATGIPARFSGSGSGTDFTLTISSLEPEDFAVYYCQQRSNWPLTFGQGTKVEIK

SEQ ID NO: 4 - protein, 119 aa, Homo sapiens
EVQLLESGGGLVQPGGSLRLSCAASGFTFSSYAMSWVRQAPGKGLEWVSAISGSGGSTYYADSVKGRFTISRDNSKNTLYLQMNSLRAEDTAVYYCAKYDGIYGELDFWGQGTLVTVSS

SEQ ID NO: 5 - protein, 10 aa, Homo sapiens
YDGIYGELDF

SEQ ID NO: 6 - protein, 115 aa, Artificial Sequence
  Concatenation of IGHV3-23*01 and IGHJ1*01
EVQLLESGGGLVQPGGSLRLSCAASGFTFSSYAMSWVRQAPGKGLEWVSAISGSGGSTYYADSVKGRFTISRDNSKNTLYLQMNSLRAEDTAVYYCAKAEYFQHWGQGTLVTVSS

SEQ ID NO: 7 - protein, 98 aa, Homo sapiens
EVQLLESGGGLVQPGGSLRLSCAASGFTFSSYAMSWVRQAPGKGLEWVSAISGSGGSTYYADSVKGRFTISRDNSKNTLYLQMNSLRAEDTAVYYCAK

SEQ ID NO: 8 - protein, 17 aa, Homo sapiens
AEYFQHWGQGTLVTVSS

SEQ ID NO: 9 - protein, 107 aa, Artificial Sequence
  Concatenation of IGKV3-11*01 and IGKJ1*01
EIVLTQSPATLSLSPGERATLSCRASQSVSSYLAWYQQKPGQAPRLLIYDASNRATGIPARFSGSGSGTDFTLTISSLEPEDFAVYYCQQRSNWPWTFGQGTKVEIK

SEQ ID NO: 10 - protein, 95 aa, Homo sapiens
EIVLTQSPATLSLSPGERATLSCRASQSVSSYLAWYQQKPGQAPRLLIYDASNRATGIPARFSGSGSGTDFTLTISSLEPEDFAVYYCQQRSNWP

SEQ ID NO: 11 - protein, 12 aa, Homo sapiens
WTFGQGTKVEIK

SEQ ID NO: 12 - protein, 119 aa, Artificial Sequence
  MSCB97 VH
EVQLLESGGGLVQPGGSLRLSCAASGFTFSSYAMSWVRQAPGKGLEWVSAISGSGGSTYYADSVKGRFTISRDNSKNTLYLQMNSLRAEDTAVYYCAKYDGCYGELDFWGQGTLVTVSS

SEQ ID NO: 13 - protein, 446 aa, Artificial Sequence
  MSCB97 HC
EVQLLESGGGLVQPGGSLRLSCAASGFTFSSYAMSWVRQAPGKGLEWVSAISGSGGSTYYADSVKGRFTISRDNSKNTLYLQMNSLRAEDTAVYYCAKYDGCYGELDFWGQGTLVTVSSASTKGPSVFPLAPCSRSTSESTAALGCLVKDYFPEPVTVSWNSGALTSGVHTFPAVLQSSGLYSLSSVVTVPSSSLGTKTYTCNVDHKPSNTKVDKRVESKYGPPCPPCPAPEAAGGPSVFLFPPKPKDTLMISRTPEVTCVVVDVSQEDPEVQFNWYVDGVEVHNAKTKPREEQFNSTYRVVSVLTVLHQDWLNGKEYKCKVSNKGLPSSIEKTISKAKGQPREPQVYTLPPSQEEMTKNQVSLTCLVKGFYPSDIAVEWESNGQPENNYKTTPPVLDSDGSFFLYSRLTVDKSRWQEGNVFSCSVMHEALHNHYTQKSLSLSLGK

SEQ ID NO: 14 - protein, 107 aa, Artificial Sequence; identical to SEQ ID NO: 3
  MSCB97 VL

SEQ ID NO: 15 - protein, 214 aa, Artificial Sequence
  MSCB97 LC
EIVLTQSPATLSLSPGERATLSCRASQSVSSYLAWYQQKPGQAPRLLIYDASNRATGIPARFSGSGSGTDFTLTISSLEPEDFAVYYCQQRSNWPLTFGQGTKVEIKRTVAAPSVFIFPPSDEQLKSGTASVVCLLNNFYPREAKVQWKVDNALQSGNSQESVTEQDSKDSTYSLSSTLTLSKADYEKHKVYACEVTHQGLSSPVTKSFNRGEC

SEQ ID NO: 16 - protein, 5 aa, Artificial Sequence
  MSCB97 HCDR1
SYAMS

SEQ ID NO: 17 - protein, 17 aa, Artificial Sequence
  MSCB97 HCDR2
AISGSGGSTYYADSVKG

SEQ ID NO: 18 - protein, 10 aa, Artificial Sequence
  MSCB97 HCDR3
YDGCYGELDF

SEQ ID NO: 19 - protein, 11 aa, Artificial Sequence
  MSCB97 LCDR1
RASQSVSSYLA

SEQ ID NO: 20 - protein, 7 aa, Artificial Sequence
  MSCB97 LCDR2
DASNRAT

SEQ ID NO: 21 - protein, 9 aa, Artificial Sequence
  MSCB97 LCDR3
QQRSNWPLT

SEQ ID NO: 22 - protein, 29 aa, Homo sapiens
HSQGTFTSDYSKYLDSRRAQDFVQWLMNT

SEQ ID NO: 23 - protein, 37 aa, Homo sapiens
HSQGTFTSDYSKYLDSRRAQDFVQWLMNTKRNRNNIA

SEQ ID NO: 24 - protein, 30 aa, Artificial Sequence
  OXM variant 1
  Xaa (2)..(2): Xaa is aminoisobutyric acid (alpha, alpha dimethylglycine)
  Lys (30)..(30): Lys with chemical modification as described in the specification
HXQGTFTSDYSKYLDERRARDFVEWLLNTK

SEQ ID NO: 25 - protein, 29 aa, Artificial Sequence
  OXM variant 2
  Xaa (2)..(2): Xaa is aminoisobutyric acid (alpha, alpha dimethylglycine)
  Lys (29)..(29): Lys with chemical modification as described in the specification
HXQGTFTSDYSKYLDERRARDFVEWLLNK

SEQ ID NO: 26 - protein, 30 aa, Artificial Sequence; identical to SEQ ID NO: 24
  OXM variant 3
  Xaa (2)..(2): Xaa is aminoisobutyric acid (alpha, alpha-dimethylglycine)
  Leu (27)..(27): Leu, wherein leu is norleucine with chemical modification as described in the specification
  Lys (30)..(30): Lys with chemical modification as described in the specification

SEQ ID NO: 27 - protein, 30 aa, Artificial Sequence; identical to SEQ ID NO: 24
  OXM variant 1/Compound 1
  Xaa (2)..(2): Xaa is aminoisobutyric acid (alpha, alpha-dimethylglycine)
  Lys (30)..(30): Lys with chemical modification as described in specification